European Patent Application EP 4 501 342 A1, published February 5, 2025. Title: Composition with antiviral, antibacterial and antifungal activity. Applicant: ELYSIUM CELL BIO ITA. The sequence listing filed with the application follows.

SEQUENCE LISTING (35 sequences)

SEQ ID NO: 1 - DNA, 24 bp, Homo sapiens
  source 1..24: mol_type = other DNA
gacccagatcatgtttgagacctt

SEQ ID NO: 2 - DNA, 21 bp, Homo sapiens
  source 1..21: mol_type = other DNA
ccagaggcgtacagggatagc

SEQ ID NO: 3 - DNA, 23 bp, Homo sapiens
  source 1..23: mol_type = other DNA
gagtgtggagaccatcaaggaag

SEQ ID NO: 4 - DNA, 24 bp, Homo sapiens
  source 1..24: mol_type = other DNA
tgctttgcgttggacattcaagtc

SEQ ID NO: 5 - DNA, 21 bp, Homo sapiens
  source 1..21: mol_type = other DNA
cctgcctaacatgcttcgaga

SEQ ID NO: 6 - DNA, 22 bp, Homo sapiens
  source 1..22: mol_type = other DNA
tgtccagctgatccttcatttg

SEQ ID NO: 7 - DNA, 21 bp, Homo sapiens
  source 1..21: mol_type = other DNA
tctctctaatcagccctctgg

SEQ ID NO: 8 - DNA, 18 bp, Homo sapiens
  source 1..18: mol_type = other DNA
gctacatgggctacaggc

SEQ ID NO: 9 - DNA, 24 bp, Homo sapiens
  source 1..24: mol_type = other DNA
caaccaacttttcgatctcttgta

SEQ ID NO: 10 - DNA, 20 bp, Homo sapiens
  source 1..20: mol_type = other DNA
tctgctcccttctgcgtaga

SEQ ID NO: 11 - DNA, 25 bp, unidentified
  source 1..25: mol_type = other DNA
  misc_feature 1: note = 5'-FAM
  misc_feature 25: note = 3'-BBQ1
acttcctcaaggaacaacattgcca

SEQ ID NO: 12 - DNA, 21 bp, unidentified
  source 1..21: mol_type = other DNA
ccctgtggttttacaccttaa

SEQ ID NO: 13 - DNA, 19 bp, unidentified
  source 1..19: mol_type = other DNA
acgattgtgcatcagctga

SEQ ID NO: 14 - DNA, 28 bp, unidentified
  source 1..28: mol_type = other DNA
  misc_feature 1: note = 5'_ROX
  misc_feature 28: note = 3'-BBQ2
ccgtctgcggtatgtggaaaggttatgg

SEQ ID NO: 15 - DNA, 26 bp, unidentified
  source 1..26: mol_type = other DNA
acaggtacgttaatagttaatagcgt

SEQ ID NO: 16 - DNA, 21 bp, unidentified
  source 1..21: mol_type = other DNA
atattgcagcagtaccacaca

SEQ ID NO: 17 - DNA, 26 bp, unidentified
  source 1..26: mol_type = other DNA
  misc_feature 1: note = 5'-CY5
  misc_feature 26: note = 3'-BBQ2
acactagccatccttactgcgcttcg

SEQ ID NO: 18 - DNA, 20 bp, unidentified
  source 1..20: mol_type = other DNA
atggcggtgtttgcagattt

SEQ ID NO: 19 - DNA, 22 bp, unidentified
  source 1..22: mol_type = other DNA
agcaacaactgaatagccaagg

SEQ ID NO: 20 - DNA, 23 bp, unidentified
  source 1..23: mol_type = other DNA
  misc_feature 1: note = 5'-HEX
  misc_feature 23: note = 3'-BHQ1
ttctgacctgaaggctctgcgcg

SEQ ID NO: 21 - DNA, 28 bp, unidentified
  source 1..28: mol_type = other DNA
aatacagccaaatccaaccaactttaca

SEQ ID NO: 22 - DNA, 21 bp, unidentified
  source 1..21: mol_type = other DNA
gccaaggaagcatgcagtaaa

SEQ ID NO: 23 - DNA, 18 bp, unidentified
  source 1..18: mol_type = other DNA
  misc_feature 1: note = 5'-FAM
  misc_feature 18: note = 3'-BHQ1
ctttagtgcacaatagca

SEQ ID NO: 24 - DNA, 20 bp, unidentified
  source 1..20: mol_type = other DNA
atggcggtgtttgcagactt

SEQ ID NO: 25 - DNA, 22 bp, unidentified
  source 1..22: mol_type = other DNA
agcaacaactgaatagccaagg

SEQ ID NO: 26 - DNA, 23 bp, unidentified
  source 1..23: mol_type = other DNA
  misc_feature 1: note = 5'-HEX
  misc_feature 23: note = 3'-BHQ1
ttctgacctgaaggctctgcgcg

SEQ ID NO: 27 - DNA, 24 bp, unidentified
  source 1..24: mol_type = other DNA
ggcaaatatggaaacatacgtgaa

SEQ ID NO: 28 - DNA, 28 bp, unidentified
  source 1..28: mol_type = other DNA
tctttttctaagacattgtattgaacag

SEQ ID NO: 29 - DNA, 27 bp, unidentified
  source 1..27: mol_type = other DNA
  misc_feature 1: note = 5'-FAM
  misc_feature 27: note = 3'-BHQ1
agcttcacgaaggctccacatacacag

SEQ ID NO: 30 - DNA, 26 bp, unidentified
  source 1..26: mol_type = other DNA
gacacaataatatttgaggcaaatgg

SEQ ID NO: 31 - DNA, 23 bp, unidentified
  source 1..23: mol_type = other DNA
gggagactgctgtttatagctcc

SEQ ID NO: 32 - DNA, 21 bp, unidentified
  source 1..21: mol_type = other DNA
  misc_feature 1: note = 5'-FAM
  misc_feature 21: note = 3'-BHQ1
gctttcgcactgagtagaggc

SEQ ID NO: 33 - DNA, 23 bp, unidentified
  source 1..23: mol_type = other DNA
cttctaaccgaggtcgaaacgta

SEQ ID NO: 34 - DNA, 25 bp, unidentified
  source 1..25: mol_type = other DNA
ggtgacaggattggtcttgtcttta

SEQ ID NO: 35 - DNA, 21 bp, unidentified
  source 1..21: mol_type = other DNA
  misc_feature 1: note = 5'-FAM
  misc_feature 21: note = 3'-BHQ1
tcaggccccctcaaagccgag